European Patent Application EP 4 632 070 A1, published October 15, 2025. Title: Protein having degrading activity of polyethylene terephthalate and method for degrading polyethylene terephthalate. Applicant: キリンホールディングス株式会社. Application WO. The sequence listing filed with the application follows.

SEQUENCE LISTING (24 sequences)

SEQ ID NO: 1 - protein, 308 aa, synthetic construct
MPITARNTLASLLLASSALLLSGTAFAANPPGGDPDPGCQTDCNYQRGPDPTDAYLEAASGPYTVSTIRVSSLVPGFGGGTIHYPTNAGGGKMAGIVVIPGYLSFESSIEWWGPRLASHGFVVMTIDTNTIYDQPSQRRDQIEAALQYLVNQSNSSSSPISGMVDSSRLAAVGWSMGGGGTLQLAADGGIKAAIALAPWNSSINDFNRIQVPTLIFACQLDAIAPVALHASPFYNRIPNTTPKAFFEMTGGDHWCANGGNIYSALLGKYGVSWMKLHLDQDTRYAPFLCGPNHAAQTLISEYRGNCPY

SEQ ID NO: 2 - DNA, 924 bp, synthetic construct
  source 1..924: mol_type = other DNA
atgccaataaccgccagaaacacactggcctcgttgctgcttgcgtcttccgcattgctgctctccggaaccgcgttcgccgccaacccgccggggggcgatcccgatcccggctgccagaccgactgcaactatcagcgcggccccgatccgaccgacgcctacctcgaagccgcgagcggaccgtacaccgtgagcaccatccgcgtttccagcctggtgcccggcttcggcggcggcaccatccactacccgaccaatgccggcggcggcaagatggctggcatcgtggtcattccgggctatctgtcgttcgagtcgtcgatcgaatggtggggaccgcggctggcttcgcacggcttcgtggtcatgaccatcgacaccaacaccatctatgaccagccgagccagcgccgcgaccagatcgaggccgccctgcagtacctggtcaaccagagcaactcctcctccagccccatcagcggcatggtcgacagctcgcgcctggcggcggtcggctggtcgatgggcggcggcgggacgctgcaactggccgccgacggcggaatcaaggccgccatcgccttggcgccatggaactccagcatcaacgacttcaaccgcatccaggtgccgaccctgatcttcgcctgccagctggatgccatcgcgccagtggccttgcatgcctcgccgttctataaccgcatcccgaacacgacccccaaggccttcttcgagatgaccggcggggaccactggtgcgccaacggcggcaacatctacagcgcgctgctcggcaagtacggcgtgtcttggatgaagctgcacctcgaccaggatacgcgttacgcgccgttcctgtgcggtcccaaccacgcggctcagaccctgatctccgaataccgaggtaactgcccgtac

SEQ ID NO: 3 - protein, 308 aa, synthetic construct
MPITARNTLASLLLASSALLLSGTAFAANPPGGDPDPGCQTDCNYQCGPDPTDAYLEAASGPYTVSTIRVSSLVPGFGGGTIHYPTNACGGKMAGIVVIPGYLSRESSIKWWGPRLASHGFVVMTIDTNTIYDQPSQRRDQIEAALQYLVNQSNSPSSPISGMVDSSRLAAVGWSMGGGATLQLAADGGIKAAIALAPWNSSINDFNRIQVPTLIFACQLDAIAPVALHASPFYNRIPNTTPKAFFEMTGGDHWCANGGNIYSALLGKYGVSWMKLHLDQDTRYAPFLCGPNHAAQPLISEYRGNCPY

SEQ ID NO: 4 - DNA, 924 bp, synthetic construct
  source 1..924: mol_type = other DNA
atgcccattacggcccgtaacactctggcttctctcctgctggcaagtagtgcactgctgctgtcaggtaccgcttttgcggcgaatccacctggtggtgatcccgatccaggctgccaaacggattgcaactaccagtgtggtcctgatcctacagatgcctacctggaagcagcgtcgggtccgtataccgtaagcacgatccgcgtgtccagtcttgtcccaggttttggcggtgggactattcactatccgaccaatgcgtgtggaggcaaaatggccggcattgtggtcattccggggtacttaagccgcgaatccagcatcaaatggtggggtccgcgtttagcgtcccacgggtttgttgtgatgaccattgacaccaacaccatctatgaccagccatctcagcgtcgcgatcagattgaagcggcgctgcagtatctggtcaatcagagcaactcaccctcgtcaccgatcagcgggatggtggactctagccgcttagctgccgtaggctggagcatgggcggcggggcaaccctgcaattggctgccgatggtggcattaaggcggcgattgccctcgcaccgtggaattcctcgattaacgactttaaccgcattcaggtgccgaccttgatctttgcatgccaacttgacgccattgctccggttgcgctgcatgcctctccgttctacaatcgcatcccgaatacgactccgaaagcgttcttcgagatgacaggcggtgaccattggtgcgcgaatggaggcaacatctacagcgcgttgctcggcaaatatggcgtttcgtggatgaaactgcaccttgatcaggatacgcggtatgccccattcctgtgtggccctaaccatgctgcacaaccgctgatcagtgagtaccgtggaaactgtccgtat

SEQ ID NO: 5 - DNA, 41 bp, synthetic construct
  source 1..41: mol_type = other DNA
aagaaggagatataccatgccaataaccgccagaaacacac

SEQ ID NO: 6 - DNA, 39 bp, synthetic construct
  source 1..39: mol_type = other DNA
gtggtggtggtggtggtacgggcagttacctcggtattc

SEQ ID NO: 7 - DNA, 27 bp, synthetic construct
  source 1..27: mol_type = other DNA
ggctataaatcgttcgagtcgtcgatc

SEQ ID NO: 8 - DNA, 27 bp, synthetic construct
  source 1..27: mol_type = other DNA
gaacgatttatagcccggaatgaccac

SEQ ID NO: 9 - DNA, 27 bp, synthetic construct
  source 1..27: mol_type = other DNA
gtgccctgcttcggcggcggcaccatc

SEQ ID NO: 10 - DNA, 27 bp, synthetic construct
  source 1..27: mol_type = other DNA
gccgaagcagggcaccaggctggaaac

SEQ ID NO: 11 - DNA, 30 bp, synthetic construct
  source 1..30: mol_type = other DNA
atcgagtgcgccctgcagtacctggtcaac

SEQ ID NO: 12 - DNA, 27 bp, synthetic construct
  source 1..27: mol_type = other DNA
cagggcgcactcgatctggtcgcggcg

SEQ ID NO: 13 - DNA, 27 bp, synthetic construct
  source 1..27: mol_type = other DNA
tatgacggcccgagccagcgccgcgac

SEQ ID NO: 14 - DNA, 28 bp, synthetic construct
  source 1..28: mol_type = other DNA
gctcgggccgtcatagatggtgttggtg

SEQ ID NO: 15 - DNA, 28 bp, synthetic construct
  source 1..28: mol_type = other DNA
ctggatatgatcgcgccagtggccttgc

SEQ ID NO: 16 - DNA, 28 bp, synthetic construct
  source 1..28: mol_type = other DNA
cgcgatcatatccagctggcaggcgaag

SEQ ID NO: 17 - DNA, 30 bp, synthetic construct
  source 1..30: mol_type = other DNA
gaccacttttgcgccaacggcggcaacatc

SEQ ID NO: 18 - DNA, 28 bp, synthetic construct
  source 1..28: mol_type = other DNA
ggcgcaaaagtggtccccgccggtcatc

SEQ ID NO: 19 - DNA, 27 bp, synthetic construct
  source 1..27: mol_type = other DNA
tgcgccgatggcggcaacatctacagc

SEQ ID NO: 20 - DNA, 25 bp, synthetic construct
  source 1..25: mol_type = other DNA
gccgccatcggcgcaccagtggtcc

SEQ ID NO: 21 - DNA, 27 bp, synthetic construct
  source 1..27: mol_type = other DNA
ggctatgattcgttcgagtcgtcgatc

SEQ ID NO: 22 - DNA, 27 bp, synthetic construct
  source 1..27: mol_type = other DNA
gaacgaatcatagcccggaatgaccac

SEQ ID NO: 23 - DNA, 23 bp, synthetic construct
  source 1..23: mol_type = other DNA
atgcccattacggcccgtaacac

SEQ ID NO: 24 - DNA, 39 bp, synthetic construct
  source 1..39: mol_type = other DNA
gtggtggtggtggtgatacggacagtttccacggtactc